European Patent Specification EP 3 885 364 B1, published June 17, 2026. Title: ANTI-CD137 ANTIBODY AND USES THEREOF. Applicant: DINGFU BIOTARGET CO., LTD. Application PCT/CN2019/105537. The sequence listing filed with the application follows.

SEQUENCE LISTING (167 sequences)

SEQ ID NO: 1 - protein, 14 aa, Artificial Sequence
  C2-WT LCDR1
TGISSDVGAYDYVS

SEQ ID NO: 2 - protein, 7 aa, Artificial Sequence
  C2-WT LCDR2
EVSKRPS

SEQ ID NO: 3 - protein, 11 aa, Artificial Sequence
  C2-WT LCDR3
SSHAGSNNFYV

SEQ ID NO: 4 - protein, 5 aa, Artificial Sequence
  C2-WT HCDR1
DYYMN

SEQ ID NO: 5 - protein, 19 aa, Artificial Sequence
  C2-WT HCDR2
YISSSASGSTIYYADSVKG

SEQ ID NO: 6 - protein, 13 aa, Artificial Sequence
  C2-WT HCDR3
VVPAGSGWRWFDP

SEQ ID NO: 7 - protein, 30 aa, Artificial Sequence
  C2-WT HFR1
EVQLVESGGGLVQPGGSLRLSCAASGFTVS

SEQ ID NO: 8 - protein, 14 aa, Artificial Sequence
  C2-WT HFR2
WIRQAPGKGLEWVS

SEQ ID NO: 9 - protein, 32 aa, Artificial Sequence
  C2-WT HFR3
RFTISRDNANNSLYLHMDSLRAEDTAIYFCAR

SEQ ID NO: 10 - protein, 11 aa, Artificial Sequence
  C2-WT HFR4
WGQGTLVTVSS

SEQ ID NO: 11 - protein, 22 aa, Artificial Sequence
  C2-WT LFR1
QSVLIQPPSASGSPGQSVTISC

SEQ ID NO: 12 - protein, 15 aa, Artificial Sequence
  C2-WT LFR2
WYQQHPGKVPKLMIY

SEQ ID NO: 13 - protein, 32 aa, Artificial Sequence
  C2-WT LFR3
GVPDRFSGSKSGDTASLTVSGLQAEDEADYYC

SEQ ID NO: 14 - protein, 10 aa, Artificial Sequence
  C2-WT LFR4
FGTGTKLTVL

SEQ ID NO: 15 - protein, 30 aa, Artificial Sequence; identical to SEQ ID NO: 7
  C2-4A HFR1

SEQ ID NO: 16 - protein, 14 aa, Artificial Sequence
  C2-4A HFR2
WIRQAPGKGLEWVS

SEQ ID NO: 17 - protein, 32 aa, Artificial Sequence
  C2-4A HFR3
RFTISRDNAKNSLYLHMDSLRAEDTAIYFCAR

SEQ ID NO: 18 - protein, 11 aa, Artificial Sequence
  C2-4A HFR4
WGQGTLVTVSS

SEQ ID NO: 19 - protein, 22 aa, Artificial Sequence
  C2-4A LFR1
QSALIQPPSASGSPGQSVTISC

SEQ ID NO: 20 - protein, 15 aa, Artificial Sequence
  C2-4A LFR2
WYQQHPGKVPKLMIY

SEQ ID NO: 21 - protein, 32 aa, Artificial Sequence
  C2-4A LFR3
GVPDRFSGSKSGNTASLTISGLQAEDEADYYC

SEQ ID NO: 22 - protein, 10 aa, Artificial Sequence
  C2-4A LFR4
FGTGTKLTVL

SEQ ID NO: 23 - protein, 30 aa, Artificial Sequence
  C2-4B HFR1
EVQLVESGGGLVQPGRSLRLSCAASGFTVS

SEQ ID NO: 24 - protein, 14 aa, Artificial Sequence
  C2-4B HFR2
WFRQAPGKGLEWVS

SEQ ID NO: 25 - protein, 32 aa, Artificial Sequence; identical to SEQ ID NO: 17
  C2-4B HFR3

SEQ ID NO: 26 - protein, 11 aa, Artificial Sequence
  C2-4B HFR4
WGQGTLVTVSS

SEQ ID NO: 27 - protein, 22 aa, Artificial Sequence
  C2-4B LFR1
QSVLIQPPSVSGSPGQSVTISC

SEQ ID NO: 28 - protein, 15 aa, Artificial Sequence
  C2-4B LFR2
WYQQHPGKVPKLMIY

SEQ ID NO: 29 - protein, 32 aa, Artificial Sequence
  C2-4B LFR3
GVPDRFSGSKSGDTASLTISGLQAEDEADYYC

SEQ ID NO: 30 - protein, 10 aa, Artificial Sequence
  C2-4B LFR4
FGTGTKLTVL

SEQ ID NO: 31 - protein, 30 aa, Artificial Sequence; identical to SEQ ID NO: 7
  C2-4C HFR1

SEQ ID NO: 32 - protein, 14 aa, Artificial Sequence
  C2-4C HFR2
WIRQAPGKGLEWVS

SEQ ID NO: 33 - protein, 32 aa, Artificial Sequence
  C2-4C HFR3
RFTISRDNAKNSLYLQMNSLRAEDTAIYFCAR

SEQ ID NO: 34 - protein, 11 aa, Artificial Sequence
  C2-4C HFR4
WGQGTLVTVSS

SEQ ID NO: 35 - protein, 22 aa, Artificial Sequence
  C2-4C LFR1
QSVLIQPPSASGSPGQSVTISC

SEQ ID NO: 36 - protein, 15 aa, Artificial Sequence
  C2-4C LFR2
WYQQHPGKVPKLMIY

SEQ ID NO: 37 - protein, 32 aa, Artificial Sequence
  C2-4C LFR3
GVPDRFSGSKSGNTASLTVSGLQAEDEADYYC

SEQ ID NO: 38 - protein, 10 aa, Artificial Sequence
  C2-4C LFR4
FGTGTKLTVL

SEQ ID NO: 39 - protein, 30 aa, Artificial Sequence; identical to SEQ ID NO: 23
  C2-5A HFR1

SEQ ID NO: 40 - protein, 14 aa, Artificial Sequence
  C2-5A HFR2
WIRQAPGKGLEWVS

SEQ ID NO: 41 - protein, 32 aa, Artificial Sequence; identical to SEQ ID NO: 17
  C2-5A HFR3

SEQ ID NO: 42 - protein, 11 aa, Artificial Sequence
  C2-5A HFR4
WGQGTLVTVSS

SEQ ID NO: 43 - protein, 22 aa, Artificial Sequence
  C2-5A LFR1
QSVLIQPPSVSGSPGQSVTISC

SEQ ID NO: 44 - protein, 15 aa, Artificial Sequence
  C2-5A LFR2
WYQQHPGKVPKLMIY

SEQ ID NO: 45 - protein, 32 aa, Artificial Sequence; identical to SEQ ID NO: 21
  C2-5A LFR3

SEQ ID NO: 46 - protein, 10 aa, Artificial Sequence
  C2-5A LFR4
FGTGTKLTVL

SEQ ID NO: 47 - protein, 30 aa, Artificial Sequence; identical to SEQ ID NO: 7
  C2-5B HFR1

SEQ ID NO: 48 - protein, 14 aa, Artificial Sequence
  C2-5B HFR2
WIRQAPGKGLEWVS

SEQ ID NO: 49 - protein, 32 aa, Artificial Sequence; identical to SEQ ID NO: 33
  C2-5B HFR3

SEQ ID NO: 50 - protein, 11 aa, Artificial Sequence
  C2-5B HFR4
WGQGTLVTVSS

SEQ ID NO: 51 - protein, 22 aa, Artificial Sequence
  C2-5B LFR1
QSVLIQPPSASGSPGQSVTISC

SEQ ID NO: 52 - protein, 15 aa, Artificial Sequence
  C2-5B LFR2
WYQQHPGKVPKLMIY

SEQ ID NO: 53 - protein, 32 aa, Artificial Sequence; identical to SEQ ID NO: 21
  C2-5B LFR3

SEQ ID NO: 54 - protein, 10 aa, Artificial Sequence
  C2-5B LFR4
FGTGTKLTVL

SEQ ID NO: 55 - protein, 30 aa, Artificial Sequence; identical to SEQ ID NO: 23
  C2-5C HFR1

SEQ ID NO: 56 - protein, 14 aa, Artificial Sequence
  C2-5C HFR2
WFRQAPGKGLEWVS

SEQ ID NO: 57 - protein, 32 aa, Artificial Sequence
  C2-5C HFR3
RFTISRDNANNSLYLHMDSLRAEDTAIYYCAR

SEQ ID NO: 58 - protein, 11 aa, Artificial Sequence
  C2-5C HFR4
WGQGTLVTVSS

SEQ ID NO: 59 - protein, 22 aa, Artificial Sequence
  C2-5C LFR1
QSVLIQPPSVSGSPGQSVTISC

SEQ ID NO: 60 - protein, 15 aa, Artificial Sequence
  C2-5C LFR2
WYQQHPGKVPKLMIY

SEQ ID NO: 61 - protein, 32 aa, Artificial Sequence; identical to SEQ ID NO: 29
  C2-5C LFR3

SEQ ID NO: 62 - protein, 10 aa, Artificial Sequence
  C2-5C LFR4
FGTGTKLTVL

SEQ ID NO: 63 - protein, 30 aa, Artificial Sequence; identical to SEQ ID NO: 7
  C2-6A HFR1

SEQ ID NO: 64 - protein, 14 aa, Artificial Sequence
  C2-6A HFR2
WIRQAPGKGLEWVS

SEQ ID NO: 65 - protein, 32 aa, Artificial Sequence; identical to SEQ ID NO: 33
  C2-6A HFR3

SEQ ID NO: 66 - protein, 11 aa, Artificial Sequence
  C2-6A HFR4
WGQGTLVTVSS

SEQ ID NO: 67 - protein, 22 aa, Artificial Sequence
  C2-6A LFR1
QSVLIQPPSVSGSPGQSVTISC

SEQ ID NO: 68 - protein, 15 aa, Artificial Sequence
  C2-6A LFR2
WYQQHPGKVPKLMIY

SEQ ID NO: 69 - protein, 32 aa, Artificial Sequence; identical to SEQ ID NO: 21
  C2-6A LFR3

SEQ ID NO: 70 - protein, 10 aa, Artificial Sequence
  C2-6A LFR4
FGTGTKLTVL

SEQ ID NO: 71 - protein, 30 aa, Artificial Sequence
  C2-6B HFR1
EVQLVESGGGLVKPGGSLRLSCAASGFTVS

SEQ ID NO: 72 - protein, 14 aa, Artificial Sequence
  C2-6B HFR2
WIRQAPGKGLEWVS

SEQ ID NO: 73 - protein, 32 aa, Artificial Sequence; identical to SEQ ID NO: 33
  C2-6B HFR3

SEQ ID NO: 74 - protein, 11 aa, Artificial Sequence
  C2-6B HFR4
WGQGTLVTVSS

SEQ ID NO: 75 - protein, 22 aa, Artificial Sequence
  C2-6B LFR1
QSVLIQPPSVSGSPGQSVTISC

SEQ ID NO: 76 - protein, 15 aa, Artificial Sequence
  C2-6B LFR2
WYQQHPGKVPKLMIY

SEQ ID NO: 77 - protein, 32 aa, Artificial Sequence; identical to SEQ ID NO: 37
  C2-6B LFR3

SEQ ID NO: 78 - protein, 10 aa, Artificial Sequence
  C2-6B LFR4
FGTGTKLTVL

SEQ ID NO: 79 - protein, 30 aa, Artificial Sequence; identical to SEQ ID NO: 71
  C2-7A HFR1

SEQ ID NO: 80 - protein, 14 aa, Artificial Sequence
  C2-7A HFR2
WIRQAPGKGLEWVS

SEQ ID NO: 81 - protein, 32 aa, Artificial Sequence; identical to SEQ ID NO: 17
  C2-7A HFR3

SEQ ID NO: 82 - protein, 11 aa, Artificial Sequence
  C2-7A HFR4
WGQGTLVTVSS

SEQ ID NO: 83 - protein, 22 aa, Artificial Sequence
  C2-7A LFR1
QSALIQPPSVSGSPGQSVTISC

SEQ ID NO: 84 - protein, 15 aa, Artificial Sequence
  C2-7A LFR2
WYQQHPGTVPKLMIY

SEQ ID NO: 85 - protein, 32 aa, Artificial Sequence; identical to SEQ ID NO: 21
  C2-7A LFR3

SEQ ID NO: 86 - protein, 10 aa, Artificial Sequence
  C2-7A LFR4
FGTGTKLTVL

SEQ ID NO: 87 - protein, 30 aa, Artificial Sequence; identical to SEQ ID NO: 71
  C2-7B HFR1

SEQ ID NO: 88 - protein, 14 aa, Artificial Sequence
  C2-7B HFR2
WIRQAPGKGLEWVS

SEQ ID NO: 89 - protein, 32 aa, Artificial Sequence
  C2-7B HFR3
RFTISRDNANNSLYLQMNSLRTEDTAIYYCAR

SEQ ID NO: 90 - protein, 11 aa, Artificial Sequence
  C2-7B HFR4
WGQGTLVTVSS

SEQ ID NO: 91 - protein, 22 aa, Artificial Sequence
  C2-7B LFR1
QSVLIQPPSVSGSPGQSVTISC

SEQ ID NO: 92 - protein, 15 aa, Artificial Sequence
  C2-7B LFR2
WYQQHPGKVPKLMIY

SEQ ID NO: 93 - protein, 32 aa, Artificial Sequence; identical to SEQ ID NO: 29
  C2-7B LFR3

SEQ ID NO: 94 - protein, 10 aa, Artificial Sequence
  C2-7B LFR4
FGTGTKLTVL

SEQ ID NO: 95 - protein, 30 aa, Artificial Sequence; identical to SEQ ID NO: 71
  C2-7BN78K HFR1

SEQ ID NO: 96 - protein, 14 aa, Artificial Sequence
  C2-7BN78K HFR2
WIRQAPGKGLEWVS

SEQ ID NO: 97 - protein, 32 aa, Artificial Sequence
  C2-7BN78K HFR3
RFTISRDNAKNSLYLQMNSLRTEDTAIYYCAR

SEQ ID NO: 98 - protein, 11 aa, Artificial Sequence
  C2-7BN78K HFR4
WGQGTLVTVSS

SEQ ID NO: 99 - protein, 22 aa, Artificial Sequence
  C2-7BN78K LFR1
QSVLIQPPSVSGSPGQSVTISC

SEQ ID NO: 100 - protein, 15 aa, Artificial Sequence
  C2-7BN78K LFR2
WYQQHPGKVPKLMIY

SEQ ID NO: 101 - protein, 32 aa, Artificial Sequence; identical to SEQ ID NO: 29
  C2-7BN78K LFR3

SEQ ID NO: 102 - protein, 10 aa, Artificial Sequence
  C2-7BN78K LFR4
FGTGTKLTVL

SEQ ID NO: 103 - protein, 111 aa, Artificial Sequence
  C2-WT VL
QSVLIQPPSASGSPGQSVTISCTGISSDVGAYDYVSWYQQHPGKVPKLMIYEVSKRPSGVPDRFSGSKSGDTASLTVSGLQAEDEADYYCSSHAGSNNFYVFGTGTKLTVL

SEQ ID NO: 104 - protein, 111 aa, Artificial Sequence
  C2-4A VL
QSALIQPPSASGSPGQSVTISCTGISSDVGAYDYVSWYQQHPGKVPKLMIYEVSKRPSGVPDRFSGSKSGNTASLTISGLQAEDEADYYCSSHAGSNNFYVFGTGTKLTVL

SEQ ID NO: 105 - protein, 111 aa, Artificial Sequence
  C2-4B VL
QSVLIQPPSVSGSPGQSVTISCTGISSDVGAYDYVSWYQQHPGKVPKLMIYEVSKRPSGVPDRFSGSKSGDTASLTISGLQAEDEADYYCSSHAGSNNFYVFGTGTKLTVL

SEQ ID NO: 106 - protein, 111 aa, Artificial Sequence
  C2-4C VL
QSVLIQPPSASGSPGQSVTISCTGISSDVGAYDYVSWYQQHPGKVPKLMIYEVSKRPSGVPDRFSGSKSGNTASLTVSGLQAEDEADYYCSSHAGSNNFYVFGTGTKLTVL

SEQ ID NO: 107 - protein, 111 aa, Artificial Sequence
  C2-5A VL
QSVLIQPPSVSGSPGQSVTISCTGISSDVGAYDYVSWYQQHPGKVPKLMIYEVSKRPSGVPDRFSGSKSGNTASLTISGLQAEDEADYYCSSHAGSNNFYVFGTGTKLTVL

SEQ ID NO: 108 - protein, 111 aa, Artificial Sequence
  C2-5B VL
QSVLIQPPSASGSPGQSVTISCTGISSDVGAYDYVSWYQQHPGKVPKLMIYEVSKRPSGVPDRFSGSKSGNTASLTISGLQAEDEADYYCSSHAGSNNFYVFGTGTKLTVL

SEQ ID NO: 109 - protein, 111 aa, Artificial Sequence; identical to SEQ ID NO: 105
  C2-5C VL

SEQ ID NO: 110 - protein, 111 aa, Artificial Sequence; identical to SEQ ID NO: 107
  C2-6A VL

SEQ ID NO: 111 - protein, 111 aa, Artificial Sequence
  C2-6B VL
QSVLIQPPSVSGSPGQSVTISCTGISSDVGAYDYVSWYQQHPGKVPKLMIYEVSKRPSGVPDRFSGSKSGNTASLTVSGLQAEDEADYYCSSHAGSNNFYVFGTGTKLTVL

SEQ ID NO: 112 - protein, 111 aa, Artificial Sequence
  C2-7A VL
QSALIQPPSVSGSPGQSVTISCTGISSDVGAYDYVSWYQQHPGTVPKLMIYEVSKRPSGVPDRFSGSKSGNTASLTISGLQAEDEADYYCSSHAGSNNFYVFGTGTKLTVL

SEQ ID NO: 113 - protein, 111 aa, Artificial Sequence; identical to SEQ ID NO: 105
  C2-7B VL

SEQ ID NO: 114 - protein, 111 aa, Artificial Sequence; identical to SEQ ID NO: 105
  C2-7BN78K VL

SEQ ID NO: 115 - DNA, 333 bp, Artificial Sequence
  C2-WT VL Nucleotide
cagtctgttctgattcagcctccctccgcgtccgggtctcctggacagtcagtcaccatctcctgcactggaatcagcagtgacgttggtgcttatgactatgtctcctggtaccaacagcacccaggcaaagtccccaaactcatgatttatgaggtcagtaagcggccctcaggggtccctgatcgcttctctggctccaagtctggcgacacggcctccctgaccgtctctgggctccaggctgaggatgaggctgattactactgcagctcacatgcaggcagcaacaatttttatgtcttcggaactgggaccaagctgaccgtccta

SEQ ID NO: 116 - DNA, 333 bp, Artificial Sequence
  C2-4A VL Nucleotide
cagagcgccctgatccagccccccagcgccagcggcagccccggccagagcgtgaccatcagctgcaccggcatcagcagcgacgtgggcgcctacgactacgtgagctggtaccagcagcaccccggcaaggtgcccaagctgatgatctacgaggtgagcaagaggcccagcggcgtgcccgacaggttcagcggcagcaagagcggcaacaccgccagcctgaccatcagcggcctgcaggccgaggacgaggccgactactactgcagcagccacgccggcagcaacaacttctacgtgttcggcaccggcaccaagctgaccgtgctg

SEQ ID NO: 117 - DNA, 333 bp, Artificial Sequence
  C2-4B VL Nucleotide
cagtccgtgctgatccagcctccttccgtgagcggaagccctggccagtccgtcaccatcagctgcaccggaatcagctccgacgtgggcgcctacgactacgtgagctggtatcaacagcaccccggcaaggtgcccaagctgatgatctacgaggtgagcaagaggcctagcggcgtgcccgacaggtttagcggcagcaagtctggtgacaccgccagcctgaccatcagcggactgcaggccgaagacgaggccgactactactgcagctcccatgccggctccaacaacttttacgtgttcggcaccggcaccaagctgacagtgctg

SEQ ID NO: 118 - DNA, 333 bp, Artificial Sequence
  C2-4C VL Nucleotide
cagagcgtgctgatccagccccccagcgccagcggcagccccggccagagcgtgaccatcagctgcaccggcatcagcagcgacgtgggcgcctacgactacgtgagctggtaccagcagcaccccggcaaggtgcccaagctgatgatctacgaggtgagcaagaggcccagcggcgtgcccgacaggttcagcggcagcaagagcggcaacaccgccagcctgaccgtgagcggcctgcaggccgaggacgaggccgactactactgcagcagccacgccggcagcaacaacttctacgtgttcggcaccggcaccaagctgaccgtgctg

SEQ ID NO: 119 - protein, 333 aa, Artificial Sequence
  C2-5A VL Nucleotide
CAGAGCGTGCTGATCCAGCCCCCCAGCGTGAGCGGCAGCCCCGGCCAGAGCGTGACCATCAGCTGCACCGGCATCAGCAGCGACGTGGGCGCCTACGACTACGTGAGCTGGTACCAGCAGCACCCCGGCAAGGTGCCCAAGCTGATGATCTACGAGGTGAGCAAGAGGCCCAGCGGCGTGCCCGACAGGTTCAGCGGCAGCAAGAGCGGCAACACCGCCAGCCTGACCATCAGCGGCCTGCAGGCCGAGGACGAGGCCGACTACTACTGCAGCAGCCACGCCGGCAGCAACAACTTCTACGTGTTCGGCACCGGCACCAAGCTGACCGTGCTG

SEQ ID NO: 120 - DNA, 333 bp, Artificial Sequence
  C2-5B VL Nucleotide
cagagcgtgctgatccagccccccagcgccagcggcagccccggccagagcgtgaccatcagctgcaccggcatcagcagcgacgtgggcgcctacgactacgtgagctggtaccagcagcaccccggcaaggtgcccaagctgatgatctacgaggtgagcaagaggcccagcggcgtgcccgacaggttcagcggcagcaagagcggcaacaccgccagcctgaccatcagcggcctgcaggccgaggacgaggccgactactactgcagcagccacgccggcagcaacaacttctacgtgttcggcaccggcaccaagctgaccgtgctg

SEQ ID NO: 121 - DNA, 333 bp, Artificial Sequence
  C2-5C VL Nucleotide
cagagcgtgctgatccagccccccagcgtgagcggcagccccggccagagcgtgaccatcagctgcaccggcatcagcagcgacgtgggcgcctacgactacgtgagctggtaccagcagcaccccggcaaggtgcccaagctgatgatctacgaggtgagcaagaggcccagcggcgtgcccgacaggttcagcggcagcaagagcggcgacaccgccagcctgaccatcagcggcctgcaggccgaggacgaggccgactactactgcagcagccacgccggcagcaacaacttctacgtgttcggcaccggcaccaagctgaccgtgctg

SEQ ID NO: 122 - DNA, 333 bp, Artificial Sequence
  C2-6A VL Nucleotide
cagagcgtgctgatccagccccccagcgtgagcggcagccccggccagagcgtgaccatcagctgcaccggcatcagcagcgacgtgggcgcctacgactacgtgagctggtaccagcagcaccccggcaaggtgcccaagctgatgatctacgaggtgagcaagaggcccagcggcgtgcccgacaggttcagcggcagcaagagcggcaacaccgccagcctgaccatcagcggcctgcaggccgaggacgaggccgactactactgcagcagccacgccggcagcaacaacttctacgtgttcggcaccggcaccaagctgaccgtgctg

SEQ ID NO: 123 - DNA, 333 bp, Artificial Sequence
  C2-6B VL Nucleotide
cagagcgtgctgatccagccccccagcgtgagcggcagccccggccagagcgtgaccatcagctgcaccggcatcagcagcgacgtgggcgcctacgactacgtgagctggtaccagcagcaccccggcaaggtgcccaagctgatgatctacgaggtgagcaagaggcccagcggcgtgcccgacaggttcagcggcagcaagagcggcaacaccgccagcctgaccgtgagcggcctgcaggccgaggacgaggccgactactactgcagcagccacgccggcagcaacaacttctacgtgttcggcaccggcaccaagctgaccgtgctg

SEQ ID NO: 124 - DNA, 333 bp, Artificial Sequence
  C2-7A VL Nucleotide
cagagcgccctgatccagcctccttccgtgagcggcagccctggacagagcgtgaccatctcctgcaccggaatcagcagcgacgtgggcgcctacgactatgtgagctggtatcaacagcaccccggaaccgtccccaagctcatgatctacgaggtgagcaagaggcccagcggagtgcccgataggttctccggcagcaaaagcggcaataccgctagcctgaccattagcggcctgcaggccgaggatgaggccgactactactgcagcagccacgccggctccaacaacttctatgtgttcggcaccggcaccaaactgaccgtgctg

SEQ ID NO: 125 - DNA, 333 bp, Artificial Sequence
  C2-7B VL Nucleotide
cagagcgtgctgattcagcctcccagcgtgagcggaagccctggacagagcgtgaccatcagctgcaccggcatcagctccgatgtgggcgcctacgactacgtgagctggtatcaacagcaccctggcaaggtgcccaagctgatgatctacgaggtgtccaaaaggcccagcggcgtgcccgataggtttagcggctccaagtccggcgacacagcctccctgaccatcagcggcctccaggctgaggatgaggccgactactactgcagcagccatgccggcagcaacaacttttacgtgttcggcaccggcacaaagctgaccgtgctg

SEQ ID NO: 126 - DNA, 333 bp, Artificial Sequence; identical to SEQ ID NO: 125
  C2-7BN78K VL Nucleotide

SEQ ID NO: 127 - protein, 124 aa, Artificial Sequence
  C2-WT VH
EVQLVESGGGLVQPGGSLRLSCAASGFTVSDYYMNWIRQAPGKGLEWVSYISSSASGSTIYYADSVKGRFTISRDNANNSLYLHMDSLRAEDTAIYFCARVVPAGSGWRWFDPWGQGTLVTVSS

SEQ ID NO: 128 - protein, 124 aa, Artificial Sequence
  C2-4A VH
EVQLVESGGGLVQPGGSLRLSCAASGFTVSDYYMNWIRQAPGKGLEWVSYISSSASGSTIYYADSVKGRFTISRDNAKNSLYLHMDSLRAEDTAIYFCARVVPAGSGWRWFDPWGQGTLVTVSS

SEQ ID NO: 129 - protein, 124 aa, Artificial Sequence
  C2-4B VH
EVQLVESGGGLVQPGRSLRLSCAASGFTVSDYYMNWFRQAPGKGLEWVSYISSSASGSTIYYADSVKGRFTISRDNANNSLYLHMDSLRAEDTAIYFCARVVPAGSGWRWFDPWGQGTLVTVSS

SEQ ID NO: 130 - protein, 124 aa, Artificial Sequence
  C2-4C VH
EVQLVESGGGLVQPGGSLRLSCAASGFTVSDYYMNWIRQAPGKGLEWVSYISSSASGSTIYYADSVKGRFTISRDNAKNSLYLQMNSLRAEDTAIYFCARVVPAGSGWRWFDPWGQGTLVTVSS

SEQ ID NO: 131 - protein, 124 aa, Artificial Sequence
  C2-5A VH
EVQLVESGGGLVQPGRSLRLSCAASGFTVSDYYMNWIRQAPGKGLEWVSYISSSASGSTIYYADSVKGRFTISRDNAKNSLYLHMDSLRAEDTAIYFCARVVPAGSGWRWFDPWGQGTLVTVSS

SEQ ID NO: 132 - protein, 124 aa, Artificial Sequence; identical to SEQ ID NO: 130
  C2-5B VH

SEQ ID NO: 133 - protein, 124 aa, Artificial Sequence
  C2-5C VH
EVQLVESGGGLVQPGRSLRLSCAASGFTVSDYYMNWFRQAPGKGLEWVSYISSSASGSTIYYADSVKGRFTISRDNANNSLYLHMDSLRAEDTAIYYCARVVPAGSGWRWFDPWGQGTLVTVSS

SEQ ID NO: 134 - protein, 124 aa, Artificial Sequence; identical to SEQ ID NO: 130
  C2-6A VH

SEQ ID NO: 135 - protein, 124 aa, Artificial Sequence
  C2-6B VH
EVQLVESGGGLVKPGGSLRLSCAASGFTVSDYYMNWIRQAPGKGLEWVSYISSSASGSTIYYADSVKGRFTISRDNAKNSLYLQMNSLRAEDTAIYFCARVVPAGSGWRWFDPWGQGTLVTVSS

SEQ ID NO: 136 - protein, 124 aa, Artificial Sequence
  C2-7A VH
EVQLVESGGGLVKPGGSLRLSCAASGFTVSDYYMNWIRQAPGKGLEWVSYISSSASGSTIYYADSVKGRFTISRDNAKNSLYLHMDSLRAEDTAIYFCARVVPAGSGWRWFDPWGQGTLVTVSS

SEQ ID NO: 137 - protein, 124 aa, Artificial Sequence
  C2-7B VH
EVQLVESGGGLVKPGGSLRLSCAASGFTVSDYYMNWIRQAPGKGLEWVSYISSSASGSTIYYADSVKGRFTISRDNANNSLYLQMNSLRTEDTAIYYCARVVPAGSGWRWFDPWGQGTLVTVSS

SEQ ID NO: 138 - protein, 124 aa, Artificial Sequence
  C2-7BN78K VH
EVQLVESGGGLVKPGGSLRLSCAASGFTVSDYYMNWIRQAPGKGLEWVSYISSSASGSTIYYADSVKGRFTISRDNAKNSLYLQMNSLRTEDTAIYYCARVVPAGSGWRWFDPWGQGTLVTVSS

SEQ ID NO: 139 - DNA, 372 bp, Artificial Sequence
  C2-WT VH Nucleotide
gaggtgcagctggtggagtctgggggaggcttggtacagcctggagggtccctgagactctcctgtgcagcctctggattcaccgtcagtgactactacatgaactggatccgccaggctccagggaagggcctggagtgggtttcatacattagtagtagtgctagtggtagtaccatatactacgcagactctgtgaagggccgattcaccatctccagggacaacgccaacaactcactgtatctgcacatggacagcctgagagccgaggacacggccatatacttctgtgcgagagtcgtcccagctggaagtgggtggaggtggttcgacccctggggccagggtaccctggtcactgtctcctca

SEQ ID NO: 140 - DNA, 372 bp, Artificial Sequence
  C2-4A VH Nucleotide
gaggtgcagctggtggagagcggcggcggcctggtgcagcccggcggcagcctgaggctgagctgcgccgccagcggcttcaccgtgagcgactactacatgaactggatcaggcaggcccccggcaagggcctggagtgggtgagctacatcagcagcagcgccagcggcagcaccatctactacgccgacagcgtgaagggcaggttcaccatcagcagggacaacgccaagaacagcctgtacctgcacatggacagcctgagggccgaggacaccgccatctacttctgcgccagggtggtgcccgccggcagcggctggaggtggttcgacccctggggccagggcaccctggtgaccgtgagcagc

SEQ ID NO: 141 - DNA, 372 bp, Artificial Sequence
  C2-4B VH Nucleotide
gaggtgcagctggtggagtccggcggaggactggtgcaacctggcagaagcctgagactgagctgtgccgccagcggcttcaccgtgtccgactactacatgaactggttcaggcaggctcccggcaagggcctggaatgggtgagctacatcagcagcagcgctagcggaagcaccatctactatgccgacagcgtgaagggcaggttcaccatcagcagggacaacgccaacaactccctgtacctgcacatggacagcctgagggccgaagacaccgccatctacttctgtgccagagtggtgcctgctggctccggctggaggtggttcgatccctggggacagggcaccctggtgaccgtgagctct

SEQ ID NO: 142 - DNA, 372 bp, Artificial Sequence
  C2-4C VH Nucleotide
gaggtgcagctggtggagagcggcggcggcctggtgcagcccggcggcagcctgaggctgagctgcgccgccagcggcttcaccgtgagcgactactacatgaactggatcaggcaggcccccggcaagggcctggagtgggtgagctacatcagcagcagcgccagcggcagcaccatctactacgccgacagcgtgaagggcaggttcaccatcagcagggacaacgccaagaacagcctgtacctgcagatgaacagcctgagggccgaggacaccgccatctacttctgcgccagggtggtgcccgccggcagcggctggaggtggttcgacccctggggccagggcaccctggtgaccgtgagcagc

SEQ ID NO: 143 - DNA, 372 bp, Artificial Sequence
  C2-5A VH Nucleotide
gaggtgcagctggtggagagcggcggcggcctggtgcagcccggcaggagcctgaggctgagctgcgccgccagcggcttcaccgtgagcgactactacatgaactggatcaggcaggcccccggcaagggcctggagtgggtgagctacatcagcagcagcgccagcggcagcaccatctactacgccgacagcgtgaagggcaggttcaccatcagcagggacaacgccaagaacagcctgtacctgcacatggacagcctgagggccgaggacaccgccatctacttctgcgccagggtggtgcccgccggcagcggctggaggtggttcgacccctggggccagggcaccctggtgaccgtgagcagc

SEQ ID NO: 144 - DNA, 372 bp, Artificial Sequence; identical to SEQ ID NO: 142
  C2-5B VH Nucleotide

SEQ ID NO: 145 - DNA, 372 bp, Artificial Sequence
  C2-5C VH Nucleotide
gaggtgcagctggtggagagcggcggcggcctggtgcagcccggcaggagcctgaggctgagctgcgccgccagcggcttcaccgtgagcgactactacatgaactggttcaggcaggcccccggcaagggcctggagtgggtgagctacatcagcagcagcgccagcggcagcaccatctactacgccgacagcgtgaagggcaggttcaccatcagcagggacaacgccaacaacagcctgtacctgcacatggacagcctgagggccgaggacaccgccatctactactgcgccagggtggtgcccgccggcagcggctggaggtggttcgacccctggggccagggcaccctggtgaccgtgagcagc

SEQ ID NO: 146 - DNA, 372 bp, Artificial Sequence; identical to SEQ ID NO: 142
  C2-6A VH Nucleotide

SEQ ID NO: 147 - DNA, 372 bp, Artificial Sequence
  C2-6B VH Nucleotide
gaggtgcagctggtggagagcggcggcggcctggtgaagcccggcggcagcctgaggctgagctgcgccgccagcggcttcaccgtgagcgactactacatgaactggatcaggcaggcccccggcaagggcctggagtgggtgagctacatcagcagcagcgccagcggcagcaccatctactacgccgacagcgtgaagggcaggttcaccatcagcagggacaacgccaagaacagcctgtacctgcagatgaacagcctgagggccgaggacaccgccatctacttctgcgccagggtggtgcccgccggcagcggctggaggtggttcgacccctggggccagggcaccctggtgaccgtgagcagc

SEQ ID NO: 148 - DNA, 372 bp, Artificial Sequence
  C2-7A VH Nucleotide
gaggtgcagctggtggaatctggtggcggactggtgaagcctggcggttctctgagactgagctgtgccgccagcggcttcaccgtgagcgactactacatgaactggatcaggcaggcccccggcaaaggcctggaatgggtgagctacatcagctcctccgcctctggttctaccatctactacgccgacagcgtgaagggcaggttcaccatcagcagggacaacgccaagaacagcctctacctgcacatggacagcctgagggccgaggacaccgctatctacttctgcgccagagtggtgcctgctggttctggctggagatggttcgatccttggggccagggcaccctggtgacagtgagcagc

SEQ ID NO: 149 - DNA, 372 bp, Artificial Sequence
  C2-7B VH Nucleotide
gaggtgcagctggtggaaagcggcggcggactggtgaagcctggaggttctctgaggctgagctgtgccgcctccggcttcaccgtgagcgactactacatgaactggatcaggcaggcccccggcaaaggactggagtgggtgagctacatctcctcctccgcctccggcagcaccatctactacgccgactccgtgaagggcaggttcaccatctccagggataacgccaacaacagcctgtacctgcagatgaactccctgaggaccgaggacaccgccatctactactgtgccagggtggtgcccgctggaagcggatggaggtggttcgacccctggggccagggaacactggtgaccgtgagcagc

SEQ ID NO: 150 - DNA, 372 bp, Artificial Sequence
  C2-7BN78K VH Nucleotide
gaggtgcagctggtggaaagcggcggcggactggtgaagcctggaggttctctgaggctgagctgtgccgcctccggcttcaccgtgagcgactactacatgaactggatcaggcaggcccccggcaaaggactggagtgggtgagctacatctcctcctccgcctccggcagcaccatctactacgccgactccgtgaagggcaggttcaccatctccagggataacgccaagaacagcctgtacctgcagatgaactccctgaggaccgaggacaccgccatctactactgtgccagggtggtgcccgctggaagcggatggaggtggttcgacccctggggccagggaacactggtgaccgtgagcagc

SEQ ID NO: 151 - protein, 489 aa, Artificial Sequence
  C2-WT-Fc
EVQLVESGGGLVQPGGSLRLSCAASGFTVSDYYMNWIRQAPGKGLEWVSYISSSASGSTIYYADSVKGRFTISRDNANNSLYLHMDSLRAEDTAIYFCARVVPAGSGWRWFDPWGQGTLVTVSSGILGSGGGGSGGGGSGGGGSQSVLIQPPSASGSPGQSVTISCTGISSDVGAYDYVSWYQQHPGKVPKLMIYEVSKRPSGVPDRFSGSKSGDTASLTVSGLQAEDEADYYCSSHAGSNNFYVFGTGTKLTVLGGGGSESKYGPPCPPCPAPEFLGGPSVFLFPPKPKDTLMISRTPEVTCVVVDVSQEDPEVQFNWYVDGVEVHNAKTKPREEQFNSTYRVVSVLTVLHQDWLNGKEYKCKVSNKGLPSSIEKTISKAKGQPREPQVYTLPPSQEEMTKNQVSLTCLVKGFYPSDIAVEWESNGQPENNYKTTPPVLDSDGSFFLYSRLTVDKSRWQEGNVFSCSVMHEALHNHYTQKSLSLSLGK

SEQ ID NO: 152 - protein, 484 aa, Artificial Sequence
  C2-4A-Fc
EVQLVESGGGLVQPGGSLRLSCAASGFTVSDYYMNWIRQAPGKGLEWVSYISSSASGSTIYYADSVKGRFTISRDNAKNSLYLHMDSLRAEDTAIYFCARVVPAGSGWRWFDPWGQGTLVTVSSGGGGSGGGGSGGGGSQSALIQPPSASGSPGQSVTISCTGISSDVGAYDYVSWYQQHPGKVPKLMIYEVSKRPSGVPDRFSGSKSGNTASLTISGLQAEDEADYYCSSHAGSNNFYVFGTGTKLTVLGGGGSESKYGPPCPPCPAPEFLGGPSVFLFPPKPKDTLMISRTPEVTCVVVDVSQEDPEVQFNWYVDGVEVHNAKTKPREEQFNSTYRVVSVLTVLHQDWLNGKEYKCKVSNKGLPSSIEKTISKAKGQPREPQVYTLPPSQEEMTKNQVSLTCLVKGFYPSDIAVEWESNGQPENNYKTTPPVLDSDGSFFLYSRLTVDKSRWQEGNVFSCSVMHEALHNHYTQKSLSLSLGK

SEQ ID NO: 153 - protein, 484 aa, Artificial Sequence
  C2-4B-Fc
EVQLVESGGGLVQPGRSLRLSCAASGFTVSDYYMNWFRQAPGKGLEWVSYISSSASGSTIYYADSVKGRFTISRDNANNSLYLHMDSLRAEDTAIYFCARVVPAGSGWRWFDPWGQGTLVTVSSGGGGSGGGGSGGGGSQSVLIQPPSVSGSPGQSVTISCTGISSDVGAYDYVSWYQQHPGKVPKLMIYEVSKRPSGVPDRFSGSKSGDTASLTISGLQAEDEADYYCSSHAGSNNFYVFGTGTKLTVLGGGGSESKYGPPCPPCPAPEFLGGPSVFLFPPKPKDTLMISRTPEVTCVVVDVSQEDPEVQFNWYVDGVEVHNAKTKPREEQFNSTYRVVSVLTVLHQDWLNGKEYKCKVSNKGLPSSIEKTISKAKGQPREPQVYTLPPSQEEMTKNQVSLTCLVKGFYPSDIAVEWESNGQPENNYKTTPPVLDSDGSFFLYSRLTVDKSRWQEGNVFSCSVMHEALHNHYTQKSLSLSLGK

SEQ ID NO: 154 - protein, 484 aa, Artificial Sequence
  C2-4C-Fc
EVQLVESGGGLVQPGGSLRLSCAASGFTVSDYYMNWIRQAPGKGLEWVSYISSSASGSTIYYADSVKGRFTISRDNAKNSLYLQMNSLRAEDTAIYFCARVVPAGSGWRWFDPWGQGTLVTVSSGGGGSGGGGSGGGGSQSVLIQPPSASGSPGQSVTISCTGISSDVGAYDYVSWYQQHPGKVPKLMIYEVSKRPSGVPDRFSGSKSGNTASLTVSGLQAEDEADYYCSSHAGSNNFYVFGTGTKLTVLGGGGSESKYGPPCPPCPAPEFLGGPSVFLFPPKPKDTLMISRTPEVTCVVVDVSQEDPEVQFNWYVDGVEVHNAKTKPREEQFNSTYRVVSVLTVLHQDWLNGKEYKCKVSNKGLPSSIEKTISKAKGQPREPQVYTLPPSQEEMTKNQVSLTCLVKGFYPSDIAVEWESNGQPENNYKTTPPVLDSDGSFFLYSRLTVDKSRWQEGNVFSCSVMHEALHNHYTQKSLSLSLGK

SEQ ID NO: 155 - protein, 484 aa, Artificial Sequence
  C2-5A-Fc
EVQLVESGGGLVQPGRSLRLSCAASGFTVSDYYMNWIRQAPGKGLEWVSYISSSASGSTIYYADSVKGRFTISRDNAKNSLYLHMDSLRAEDTAIYFCARVVPAGSGWRWFDPWGQGTLVTVSSGGGGSGGGGSGGGGSQSVLIQPPSVSGSPGQSVTISCTGISSDVGAYDYVSWYQQHPGKVPKLMIYEVSKRPSGVPDRFSGSKSGNTASLTISGLQAEDEADYYCSSHAGSNNFYVFGTGTKLTVLGGGGSESKYGPPCPPCPAPEFLGGPSVFLFPPKPKDTLMISRTPEVTCVVVDVSQEDPEVQFNWYVDGVEVHNAKTKPREEQFNSTYRVVSVLTVLHQDWLNGKEYKCKVSNKGLPSSIEKTISKAKGQPREPQVYTLPPSQEEMTKNQVSLTCLVKGFYPSDIAVEWESNGQPENNYKTTPPVLDSDGSFFLYSRLTVDKSRWQEGNVFSCSVMHEALHNHYTQKSLSLSLGK

SEQ ID NO: 156 - protein, 484 aa, Artificial Sequence
  C2-5B-Fc
EVQLVESGGGLVQPGGSLRLSCAASGFTVSDYYMNWIRQAPGKGLEWVSYISSSASGSTIYYADSVKGRFTISRDNAKNSLYLQMNSLRAEDTAIYFCARVVPAGSGWRWFDPWGQGTLVTVSSGGGGSGGGGSGGGGSQSVLIQPPSASGSPGQSVTISCTGISSDVGAYDYVSWYQQHPGKVPKLMIYEVSKRPSGVPDRFSGSKSGNTASLTISGLQAEDEADYYCSSHAGSNNFYVFGTGTKLTVLGGGGSESKYGPPCPPCPAPEFLGGPSVFLFPPKPKDTLMISRTPEVTCVVVDVSQEDPEVQFNWYVDGVEVHNAKTKPREEQFNSTYRVVSVLTVLHQDWLNGKEYKCKVSNKGLPSSIEKTISKAKGQPREPQVYTLPPSQEEMTKNQVSLTCLVKGFYPSDIAVEWESNGQPENNYKTTPPVLDSDGSFFLYSRLTVDKSRWQEGNVFSCSVMHEALHNHYTQKSLSLSLGK

SEQ ID NO: 157 - protein, 484 aa, Artificial Sequence
  C2-5C-Fc
EVQLVESGGGLVQPGRSLRLSCAASGFTVSDYYMNWFRQAPGKGLEWVSYISSSASGSTIYYADSVKGRFTISRDNANNSLYLHMDSLRAEDTAIYYCARVVPAGSGWRWFDPWGQGTLVTVSSGGGGSGGGGSGGGGSQSVLIQPPSVSGSPGQSVTISCTGISSDVGAYDYVSWYQQHPGKVPKLMIYEVSKRPSGVPDRFSGSKSGDTASLTISGLQAEDEADYYCSSHAGSNNFYVFGTGTKLTVLGGGGSESKYGPPCPPCPAPEFLGGPSVFLFPPKPKDTLMISRTPEVTCVVVDVSQEDPEVQFNWYVDGVEVHNAKTKPREEQFNSTYRVVSVLTVLHQDWLNGKEYKCKVSNKGLPSSIEKTISKAKGQPREPQVYTLPPSQEEMTKNQVSLTCLVKGFYPSDIAVEWESNGQPENNYKTTPPVLDSDGSFFLYSRLTVDKSRWQEGNVFSCSVMHEALHNHYTQKSLSLSLGK

SEQ ID NO: 158 - protein, 484 aa, Artificial Sequence
  C2-6A-Fc
EVQLVESGGGLVQPGGSLRLSCAASGFTVSDYYMNWIRQAPGKGLEWVSYISSSASGSTIYYADSVKGRFTISRDNAKNSLYLQMNSLRAEDTAIYFCARVVPAGSGWRWFDPWGQGTLVTVSSGGGGSGGGGSGGGGSQSVLIQPPSVSGSPGQSVTISCTGISSDVGAYDYVSWYQQHPGKVPKLMIYEVSKRPSGVPDRFSGSKSGNTASLTISGLQAEDEADYYCSSHAGSNNFYVFGTGTKLTVLGGGGSESKYGPPCPPCPAPEFLGGPSVFLFPPKPKDTLMISRTPEVTCVVVDVSQEDPEVQFNWYVDGVEVHNAKTKPREEQFNSTYRVVSVLTVLHQDWLNGKEYKCKVSNKGLPSSIEKTISKAKGQPREPQVYTLPPSQEEMTKNQVSLTCLVKGFYPSDIAVEWESNGQPENNYKTTPPVLDSDGSFFLYSRLTVDKSRWQEGNVFSCSVMHEALHNHYTQKSLSLSLGK

SEQ ID NO: 159 - protein, 484 aa, Artificial Sequence
  C2-6B-Fc
EVQLVESGGGLVKPGGSLRLSCAASGFTVSDYYMNWIRQAPGKGLEWVSYISSSASGSTIYYADSVKGRFTISRDNAKNSLYLQMNSLRAEDTAIYFCARVVPAGSGWRWFDPWGQGTLVTVSSGGGGSGGGGSGGGGSQSVLIQPPSVSGSPGQSVTISCTGISSDVGAYDYVSWYQQHPGKVPKLMIYEVSKRPSGVPDRFSGSKSGNTASLTVSGLQAEDEADYYCSSHAGSNNFYVFGTGTKLTVLGGGGSESKYGPPCPPCPAPEFLGGPSVFLFPPKPKDTLMISRTPEVTCVVVDVSQEDPEVQFNWYVDGVEVHNAKTKPREEQFNSTYRVVSVLTVLHQDWLNGKEYKCKVSNKGLPSSIEKTISKAKGQPREPQVYTLPPSQEEMTKNQVSLTCLVKGFYPSDIAVEWESNGQPENNYKTTPPVLDSDGSFFLYSRLTVDKSRWQEGNVFSCSVMHEALHNHYTQKSLSLSLGK

SEQ ID NO: 160 - protein, 484 aa, Artificial Sequence
  C2-7A-Fc
EVQLVESGGGLVKPGGSLRLSCAASGFTVSDYYMNWIRQAPGKGLEWVSYISSSASGSTIYYADSVKGRFTISRDNAKNSLYLHMDSLRAEDTAIYFCARVVPAGSGWRWFDPWGQGTLVTVSSGGGGSGGGGSGGGGSQSALIQPPSVSGSPGQSVTISCTGISSDVGAYDYVSWYQQHPGTVPKLMIYEVSKRPSGVPDRFSGSKSGNTASLTISGLQAEDEADYYCSSHAGSNNFYVFGTGTKLTVLGGGGSESKYGPPCPPCPAPEFLGGPSVFLFPPKPKDTLMISRTPEVTCVVVDVSQEDPEVQFNWYVDGVEVHNAKTKPREEQFNSTYRVVSVLTVLHQDWLNGKEYKCKVSNKGLPSSIEKTISKAKGQPREPQVYTLPPSQEEMTKNQVSLTCLVKGFYPSDIAVEWESNGQPENNYKTTPPVLDSDGSFFLYSRLTVDKSRWQEGNVFSCSVMHEALHNHYTQKSLSLSLGK

SEQ ID NO: 161 - protein, 484 aa, Artificial Sequence
  C2-7B-Fc
EVQLVESGGGLVKPGGSLRLSCAASGFTVSDYYMNWIRQAPGKGLEWVSYISSSASGSTIYYADSVKGRFTISRDNANNSLYLQMNSLRTEDTAIYYCARVVPAGSGWRWFDPWGQGTLVTVSSGGGGSGGGGSGGGGSQSVLIQPPSVSGSPGQSVTISCTGISSDVGAYDYVSWYQQHPGKVPKLMIYEVSKRPSGVPDRFSGSKSGDTASLTISGLQAEDEADYYCSSHAGSNNFYVFGTGTKLTVLGGGGSESKYGPPCPPCPAPEFLGGPSVFLFPPKPKDTLMISRTPEVTCVVVDVSQEDPEVQFNWYVDGVEVHNAKTKPREEQFNSTYRVVSVLTVLHQDWLNGKEYKCKVSNKGLPSSIEKTISKAKGQPREPQVYTLPPSQEEMTKNQVSLTCLVKGFYPSDIAVEWESNGQPENNYKTTPPVLDSDGSFFLYSRLTVDKSRWQEGNVFSCSVMHEALHNHYTQKSLSLSLGK

SEQ ID NO: 162 - protein, 484 aa, Artificial Sequence
  C2-7BN78K-Fc
EVQLVESGGGLVKPGGSLRLSCAASGFTVSDYYMNWIRQAPGKGLEWVSYISSSASGSTIYYADSVKGRFTISRDNAKNSLYLQMNSLRTEDTAIYYCARVVPAGSGWRWFDPWGQGTLVTVSSGGGGSGGGGSGGGGSQSVLIQPPSVSGSPGQSVTISCTGISSDVGAYDYVSWYQQHPGKVPKLMIYEVSKRPSGVPDRFSGSKSGDTASLTISGLQAEDEADYYCSSHAGSNNFYVFGTGTKLTVLGGGGSESKYGPPCPPCPAPEFLGGPSVFLFPPKPKDTLMISRTPEVTCVVVDVSQEDPEVQFNWYVDGVEVHNAKTKPREEQFNSTYRVVSVLTVLHQDWLNGKEYKCKVSNKGLPSSIEKTISKAKGQPREPQVYTLPPSQEEMTKNQVSLTCLVKGFYPSDIAVEWESNGQPENNYKTTPPVLDSDGSFFLYSRLTVDKSRWQEGNVFSCSVMHEALHNHYTQKSLSLSLGK

SEQ ID NO: 163 - protein, 229 aa, Artificial Sequence
  Fc
ESKYGPPCPPCPAPEFLGGPSVFLFPPKPKDTLMISRTPEVTCVVVDVSQEDPEVQFNWYVDGVEVHNAKTKPREEQFNSTYRVVSVLTVLHQDWLNGKEYKCKVSNKGLPSSIEKTISKAKGQPREPQVYTLPPSQEEMTKNQVSLTCLVKGFYPSDIAVEWESNGQPENNYKTTPPVLDSDGSFFLYSRLTVDKSRWQEGNVFSCSVMHEALHNHYTQKSLSLSLGK

SEQ ID NO: 164 - protein, 229 aa, Artificial Sequence
  Fc-WT
ESKYGPPCPSCPAPEFLGGPSVFLFPPKPKDTLMISRTPEVTCVVVDVSQEDPEVQFNWYVDGVEVHNAKTKPREEQFNSTYRVVSVLTVLHQDWLNGKEYKCKVSNKGLPSSIEKTISKAKGQPREPQVYTLPPSQEEMTKNQVSLTCLVKGFYPSDIAVEWESNGQPENNYKTTPPVLDSDGSFFLYSRLTVDKSRWQEGNVFSCSVMHEALHNHYTQKSLSLSLGK

SEQ ID NO: 165 - protein, 15 aa, Artificial Sequence
  (G4S)3
GGGGSGGGGSGGGGS

SEQ ID NO: 166 - protein, 5 aa, Artificial Sequence
  G4S
GGGGS

SEQ ID NO: 167 - DNA, 1452 bp, Artificial Sequence
  C2-7BN78K-Fc Nucleotide
gaggtgcagctggtggaaagcggcggcggactggtgaagcctggaggttctctgaggctgagctgtgccgcctccggcttcaccgtgagcgactactacatgaactggatcaggcaggcccccggcaaaggactggagtgggtgagctacatctcctcctccgcctccggcagcaccatctactacgccgactccgtgaagggcaggttcaccatctccagggataacgccaagaacagcctgtacctgcagatgaactccctgaggaccgaggacaccgccatctactactgtgccagggtggtgcccgctggaagcggatggaggtggttcgacccctggggccagggaacactggtgaccgtgagcagcggaggaggaggaagcggaggaggaggaagcggaggaggcggcagccagagcgtgctgattcagcctcccagcgtgagcggaagccctggacagagcgtgaccatcagctgcaccggcatcagctccgatgtgggcgcctacgactacgtgagctggtatcaacagcaccctggcaaggtgcccaagctgatgatctacgaggtgtccaaaaggcccagcggcgtgcccgataggtttagcggctccaagtccggcgacacagcctccctgaccatcagcggcctccaggctgaggatgaggccgactactactgcagcagccatgccggcagcaacaacttttacgtgttcggcaccggcacaaagctgaccgtgctgggcggaggcggcagcgagtccaaatatggtcccccatgcccaccatgcccagctccggagttcctggggggaccatcagtcttcctgttccccccaaaacccaaggacactctcatgatctcccggacccctgaggtcacgtgcgtggtggtggacgtgagccaggaagaccccgaggtccagttcaactggtacgtggatggcgtggaggtgcataatgccaagacaaagccgcgggaggagcagttcaacagcacgtaccgtgtggtcagcgtcctcaccgtcctgcaccaggactggctgaacggcaaggagtacaagtgcaaggtctccaacaaaggcctcccgtcctccatcgagaaaaccatctccaaagccaaagggcagccccgagagccacaggtgtacaccctgcccccatcccaggaggagatgaccaagaaccaggtcagcctgacctgcctggtcaaaggcttctaccccagcgacatcgccgtggagtgggagagcaatgggcagccggagaacaactacaagaccacgcctcccgtgctggactccgacggctccttcttcctctacagcaggctaaccgtggacaagagcaggtggcaggaggggaatgtcttctcatgctccgtgatgcatgaggctctgcacaaccactacacacagaagagcctctccctgtctctgggtaaa